European Patent Specification EP 3 782 603 B1, published November 22, 2023. Title: PHARMACEUTICAL COMPOSITION AND KIT FOR TREATING GOUT. Applicant: UNIVERSITY-INDUSTRY FOUNDATION(UIF), YONSEI UNIVERSITY. The sequence listing filed with the application follows.

SEQUENCE LISTING (5 sequences)

SEQ ID NO: 1 - protein, 15 aa, Artificial Sequence
  peptide 1
ARGVNPGIMGRDYWG

SEQ ID NO: 2 - protein, 15 aa, Artificial Sequence
  peptide 2
ARYAGSLESGADDWG

SEQ ID NO: 3 - protein, 15 aa, Artificial Sequence
  peptide 3
ARCESGRPGSVDFWG

SEQ ID NO: 4 - protein, 15 aa, Artificial Sequence
  peptide 4
ARCLELLGRKIDFWG

SEQ ID NO: 5 - protein, 15 aa, Artificial Sequence
  peptide 5
ARCLELLGRKIDFWG